European Patent Application EP 4 177 335 A1, published May 10, 2023. Title: METHODS FOR THE IN VITRO MANUFACTURE OF GASTRIC FUNDUS TISSUE AND COMPOSITIONS RELATED TO SAME. Applicant: Children's Hopital Medical Center. Application EP 22189427.2, filed August 9, 2022. The sequence listing filed with the application follows.

SEQUENCE LISTING (64 sequences)

SEQ ID NO: 1 - DNA, 20 bp, synthetic construct
  misc_feature 1..20: note = hATP4A forward
  source 1..20: mol_type = other DNA
tggtagtagccaaagcagcc

SEQ ID NO: 2 - DNA, 19 bp, synthetic construct
  misc_feature 1..19: note = hATP4A reverse
  source 1..19: mol_type = other DNA
tgccatccaggctagtgag

SEQ ID NO: 3 - DNA, 20 bp, synthetic construct
  misc_feature 1..20: note = hATP4B forward
  source 1..20: mol_type = other DNA
accacgtagaaggccacgta

SEQ ID NO: 4 - DNA, 20 bp, synthetic construct
  misc_feature 1..20: note = hATP4B reverse
  source 1..20: mol_type = other DNA
tggaggagttccagcgttac

SEQ ID NO: 5 - DNA, 20 bp, synthetic construct
  misc_feature 1..20: note = hAXIN2 forward
  source 1..20: mol_type = other DNA
ctggtgcaaagacatagcca

SEQ ID NO: 6 - DNA, 20 bp, synthetic construct
  misc_feature 1..20: note = hAXIN2 reverse
  source 1..20: mol_type = other DNA
agtgtgaggtccacggaaac

SEQ ID NO: 7 - DNA, 20 bp, synthetic construct
  misc_feature 1..20: note = hCCK forward
  source 1..20: mol_type = other DNA
cggtcacttatcctgtggct

SEQ ID NO: 8 - DNA, 20 bp, synthetic construct
  misc_feature 1..20: note = hCCK reverse
  source 1..20: mol_type = other DNA
ctgcgaagatcaatccagca

SEQ ID NO: 9 - DNA, 22 bp, synthetic construct
  misc_feature 1..22: note = hCDX2 forward
  source 1..22: mol_type = other DNA
ctggagctggagaaggagtttc

SEQ ID NO: 10 - DNA, 24 bp, synthetic construct
  misc_feature 1..24: note = hCDX2 reverse
  source 1..24: mol_type = other DNA
attttaacctgcctctcagagagc

SEQ ID NO: 11 - DNA, 20 bp, synthetic construct
  misc_feature 1..20: note = hCHGA forward
  source 1..20: mol_type = other DNA
tgacctcaacgatgcatttc

SEQ ID NO: 12 - DNA, 20 bp, synthetic construct
  misc_feature 1..20: note = hCHGA reverse
  source 1..20: mol_type = other DNA
ctgtcctggctcttctgctc

SEQ ID NO: 13 - DNA, 21 bp, synthetic construct
  misc_feature 1..21: note = hGAPDH forward
  source 1..21: mol_type = other DNA
cccatcaccatcttccaggag

SEQ ID NO: 14 - DNA, 22 bp, synthetic construct
  misc_feature 1..22: note = hGAPDH reverse
  source 1..22: mol_type = other DNA
cttctccatggtggtgaagacg

SEQ ID NO: 15 - DNA, 20 bp, synthetic construct
  misc_feature 1..20: note = hGAST reverse
  source 1..20: mol_type = other DNA
cagagccagtgcaaagatca

SEQ ID NO: 16 - DNA, 20 bp, synthetic construct
  misc_feature 1..20: note = hGAST reverse
  source 1..20: mol_type = other DNA
agagacctgagaggcaccag

SEQ ID NO: 17 - DNA, 21 bp, synthetic construct
  misc_feature 1..21: note = hGATA4 forward
  source 1..21: mol_type = other DNA
tccaaaccagaaaacggaagc

SEQ ID NO: 18 - DNA, 20 bp, synthetic construct
  misc_feature 1..20: note = hGATA4 reverse
  source 1..20: mol_type = other DNA
gcccgtagtgagatgacagg

SEQ ID NO: 19 - DNA, 20 bp, synthetic construct
  misc_feature 1..20: note = hGHRL forward
  source 1..20: mol_type = other DNA
gctggtactgaacccctgac

SEQ ID NO: 20 - DNA, 20 bp, synthetic construct
  misc_feature 1..20: note = hGHRL reverse
  source 1..20: mol_type = other DNA
gatggaggtcaagcagaagg

SEQ ID NO: 21 - DNA, 20 bp, synthetic construct
  misc_feature 1..20: note = hGIF forward
  source 1..20: mol_type = other DNA
cattttccgcgatattgttg

SEQ ID NO: 22 - DNA, 20 bp, synthetic construct
  misc_feature 1..20: note = hGIF reverse
  source 1..20: mol_type = other DNA
gcacagcgcaaaaatcctat

SEQ ID NO: 23 - DNA, 17 bp, synthetic construct
  misc_feature 1..17: note = hIRX2 forward
  source 1..17: mol_type = other DNA
gtggtgtgcgcgtcgta

SEQ ID NO: 24 - DNA, 17 bp, synthetic construct
  misc_feature 1..17: note = hIRX2 reverse
  source 1..17: mol_type = other DNA
ggcgttcagcccctacc

SEQ ID NO: 25 - DNA, 20 bp, synthetic construct
  misc_feature 1..20: note = hIRX3 forward
  source 1..20: mol_type = other DNA
ggagagagccgataagacca

SEQ ID NO: 26 - DNA, 20 bp, synthetic construct
  misc_feature 1..20: note = hIRX3 reverse
  source 1..20: mol_type = other DNA
agtgccttggaagtggagaa

SEQ ID NO: 27 - DNA, 20 bp, synthetic construct
  misc_feature 1..20: note = hIRX5 forward
  source 1..20: mol_type = other DNA
ggtgtgtggtcgtagggaga

SEQ ID NO: 28 - DNA, 19 bp, synthetic construct
  misc_feature 1..19: note = hIRX5 reverse
  source 1..19: mol_type = other DNA
gctacaactcgcacctcca

SEQ ID NO: 29 - DNA, 19 bp, synthetic construct
  misc_feature 1..19: note = hMIST1 forward
  source 1..19: mol_type = other DNA
tgctggacatggtcaggat

SEQ ID NO: 30 - DNA, 20 bp, synthetic construct
  misc_feature 1..20: note = hMIST1 reverse
  source 1..20: mol_type = other DNA
cggacaagaagctctccaag

SEQ ID NO: 31 - DNA, 20 bp, synthetic construct
  misc_feature 1..20: note = hMUC2 forward
  source 1..20: mol_type = other DNA
tgtaggcatcgctcttctca

SEQ ID NO: 32 - DNA, 20 bp, synthetic construct
  misc_feature 1..20: note = hMUC2 reverse
  source 1..20: mol_type = other DNA
gacaccatctacctcacccg

SEQ ID NO: 33 - DNA, 20 bp, synthetic construct
  misc_feature 1..20: note = hMUC5AC forward
  source 1..20: mol_type = other DNA
ccaaggagaacctcccatat

SEQ ID NO: 34 - DNA, 18 bp, synthetic construct
  misc_feature 1..18: note = hMUC5AC reverse
  source 1..18: mol_type = other DNA
ccaagcgtcattcctgag

SEQ ID NO: 35 - DNA, 24 bp, synthetic construct
  misc_feature 1..24: note = hMUC6 forward
  source 1..24: mol_type = other DNA
cagcaggaggagatcacgttcaag

SEQ ID NO: 36 - DNA, 24 bp, synthetic construct
  misc_feature 1..24: note = hMUC6 reverse
  source 1..24: mol_type = other DNA
gtgggtgttttcctgtctgtcatc

SEQ ID NO: 37 - DNA, 18 bp, synthetic construct
  misc_feature 1..18: note = hPDX1 forward
  source 1..18: mol_type = other DNA
cgtccgcttgttctcctc

SEQ ID NO: 38 - DNA, 20 bp, synthetic construct
  misc_feature 1..20: note = hPDX1 reverse
  source 1..20: mol_type = other DNA
cctttcccatggatgaagtc

SEQ ID NO: 39 - DNA, 20 bp, synthetic construct
  misc_feature 1..20: note = hSCT forward
  source 1..20: mol_type = other DNA
ggttctgaaaccataggccc

SEQ ID NO: 40 - DNA, 18 bp, synthetic construct
  misc_feature 1..18: note = hSCT reverse
  source 1..18: mol_type = other DNA
gtcagggtccaacatgcc

SEQ ID NO: 41 - DNA, 20 bp, synthetic construct
  misc_feature 1..20: note = hSOX2 forward
  source 1..20: mol_type = other DNA
gcttagcctcgtcgatgaac

SEQ ID NO: 42 - DNA, 20 bp, synthetic construct
  misc_feature 1..20: note = hSOX2 reverse
  source 1..20: mol_type = other DNA
aaccccaagatgcacaactc

SEQ ID NO: 43 - DNA, 20 bp, synthetic construct
  misc_feature 1..20: note = mCdx2 forward
  source 1..20: mol_type = other DNA
tctgtgtacaccacccggta

SEQ ID NO: 44 - DNA, 20 bp, synthetic construct
  misc_feature 1..20: note = mCdx2 reverse
  source 1..20: mol_type = other DNA
gaaacctgtgcgagtggatg

SEQ ID NO: 45 - DNA, 18 bp, synthetic construct
  misc_feature 1..18: note = mGata4 forward
  source 1..18: mol_type = other DNA
ccatctcgcctccagagt

SEQ ID NO: 46 - DNA, 20 bp, synthetic construct
  misc_feature 1..20: note = mGata4 reverse
  source 1..20: mol_type = other DNA
ctggaagacaccccaatctc

SEQ ID NO: 47 - DNA, 20 bp, synthetic construct
  misc_feature 1..20: note = mGapdh forward
  source 1..20: mol_type = other DNA
ttgatggcaacaatctccac

SEQ ID NO: 48 - DNA, 20 bp, synthetic construct
  misc_feature 1..20: note = mGapdh reverse
  source 1..20: mol_type = other DNA
cgtcccgtagacaaaatggt

SEQ ID NO: 49 - DNA, 20 bp, synthetic construct
  misc_feature 1..20: note = mIrx1 forward
  source 1..20: mol_type = other DNA
aataagcaggcgttgtgtgg

SEQ ID NO: 50 - DNA, 20 bp, synthetic construct
  misc_feature 1..20: note = mIrx1 reverse
  source 1..20: mol_type = other DNA
ctcagcctcttctcgcagat

SEQ ID NO: 51 - DNA, 19 bp, synthetic construct
  misc_feature 1..19: note = mIrx2 forward
  source 1..19: mol_type = other DNA
agctggtatggataggccg

SEQ ID NO: 52 - DNA, 18 bp, synthetic construct
  misc_feature 1..18: note = mIrx2 reverse
  source 1..18: mol_type = other DNA
ggcttcccgtcctacgtg

SEQ ID NO: 53 - DNA, 20 bp, synthetic construct
  misc_feature 1..20: note = mIrx3 reverse
  source 1..20: mol_type = other DNA
ataagaccagagcagcgtcc

SEQ ID NO: 54 - DNA, 20 bp, synthetic construct
  misc_feature 1..20: note = mIrx3 reverse
  source 1..20: mol_type = other DNA
gtgccttggaagtggagaaa

SEQ ID NO: 55 - DNA, 20 bp, synthetic construct
  misc_feature 1..20: note = mIrx5 forward
  source 1..20: mol_type = other DNA
ggagtgtggtcgtagggaga

SEQ ID NO: 56 - DNA, 19 bp, synthetic construct
  misc_feature 1..19: note = mIrx5 reverse
  source 1..19: mol_type = other DNA
gctacaactcgcacctcca

SEQ ID NO: 57 - DNA, 20 bp, synthetic construct
  misc_feature 1..20: note = mPdx1 forward
  source 1..20: mol_type = other DNA
acgggtcctcttgttttcct

SEQ ID NO: 58 - DNA, 20 bp, synthetic construct
  misc_feature 1..20: note = mPdx1 reverse
  source 1..20: mol_type = other DNA
tggatgaaatccaccaaagc

SEQ ID NO: 59 - DNA, 18 bp, synthetic construct
  misc_feature 1..18: note = mPitx1 forward
  source 1..18: mol_type = other DNA
gtccatggaggtggggac

SEQ ID NO: 60 - DNA, 19 bp, synthetic construct
  misc_feature 1..19: note = mPitx1 reverse
  source 1..19: mol_type = other DNA
gcttaggcgccactctctt

SEQ ID NO: 61 - DNA, 20 bp, synthetic construct
  misc_feature 1..20: note = mSox2 forward
  source 1..20: mol_type = other DNA
aaagcgttaatttggatggg

SEQ ID NO: 62 - DNA, 20 bp, synthetic construct
  misc_feature 1..20: note = mSox2 reverse
  source 1..20: mol_type = other DNA
acaagagaattgggaggggt

SEQ ID NO: 63 - DNA, 20 bp, synthetic construct
  misc_feature 1..20: note = mTrp63 forward
  source 1..20: mol_type = other DNA
agcttcttcagttcggtgga

SEQ ID NO: 64 - DNA, 20 bp, synthetic construct
  misc_feature 1..20: note = mTrp63 reverse
  source 1..20: mol_type = other DNA
cctccaacacagattacccg